European Patent Application EP 4 431 593 A1, published September 18, 2024. Title: Novel strain of Schizochytrium sp. with easy intracellular oil extraction and a method for producing oil containing omega3 using the same. Applicant: 씨제이제일제당 (주). The sequence listing filed with the application follows.

SEQUENCE LISTING (3 sequences)

SEQ ID NO: 1 - DNA, 850 bp, synthetic construct
  misc_feature 1..850: note = 18s rRNA sequence of CD01-1821
  source 1..850: mol_type = other DNA
aagcttgtttcaaagattaccatgcatgtgtaagtataagcgattgtactgtgagactgcgaacggctcattatatcagtaataatttcttcggtagtttcttttataggatacctgcagtaattctggaaataatacatgctgtaagagccctgtatggggctgcacttattagattgaagccgattttattggtgaatcatgataattgagcagattgacttttttgtcatgaatcgtttgagtttctgccccatcagttgtcacggtagtgtattggactacggtgactataacgggtgacggaagttagggctgactccggaagggagcctgaaacggctaccatatccaaggatagcacaggccgtaaattacccactgtggactccacaggtagtgacagaaatatcgatgcaagcgtgtatgcgttttgctatcggaatgaagcaatgtaaaaccctcatcgaggatcaactggagggcaagtctggtgccagcagccgcggtaattccagctccagaagcatatgctaaagttgttgcagttaaaaagctgtagttgaattttggcatgggcaccggtgctttccctgaatggggattgattgttgtgttgccttggccatctttttcttcttttttggaatctttcactgtaatcaaagcaagtgttccaagcaggcgatgaccggtatgtttattatgggatgataaataggacttgggtgctattttgttggtttgcacgcctgagtaaggttaataggaacagttgggggtattcgtatttaggagctagaggtgaaattcttgattccaaaagacaaacagaggaaaggcattccca

SEQ ID NO: 2 - DNA, 21 bp, synthetic construct
  misc_feature 1..21: note = Synthetic_18S Fwd primer
  source 1..21: mol_type = other DNA
aacctggttgatcctgccagt

SEQ ID NO: 3 - DNA, 18 bp, synthetic construct
  misc_feature 1..18: note = Synthetic_LABY-ARev primer
  source 1..18: mol_type = other DNA
gggatcgaagatgattag